European Patent Application EP 4 635 985 A1, published October 22, 2025. Title: ANTI-TM4SF4 HUMANIZED ANTIBODIES AND USE THEREOF. Applicant: KOREA ATOMIC ENERGY RESEARCH INSTITUTE. Application KR. The sequence listing filed with the application follows.

SEQUENCE LISTING (20 sequences)

SEQ ID NO: 1 - protein, 30 aa, synthetic construct
EITLKESGPTLVKPTQTLTLTCTFSGFSLS

SEQ ID NO: 2 - protein, 14 aa, synthetic construct
WIRQPPGKALEWLA

SEQ ID NO: 3 - protein, 32 aa, synthetic construct
RLTITKDTSKNQVVLTMTNMDPVDTATYYCAR

SEQ ID NO: 4 - protein, 11 aa, synthetic construct
WGQGTLVTVSS

SEQ ID NO: 5 - protein, 23 aa, synthetic construct
DIVMTQSPDSLAVSLGERATINC

SEQ ID NO: 6 - protein, 15 aa, synthetic construct
WYQQKPGQPPKLLIY

SEQ ID NO: 7 - protein, 32 aa, synthetic construct
GVPDRFSGSGSGTDFTLTISLMQAEDVAVYYC

SEQ ID NO: 8 - protein, 10 aa, synthetic construct
FGQGTKVEIK

SEQ ID NO: 9 - protein, 7 aa, synthetic construct
TYGIGVS

SEQ ID NO: 10 - protein, 16 aa, synthetic construct
HIWWNDNKYYNTALKS

SEQ ID NO: 11 - protein, 10 aa, synthetic construct
KEGSSAPFAY

SEQ ID NO: 12 - protein, 17 aa, synthetic construct
KSSQSLLNSSNQKNYLA

SEQ ID NO: 13 - protein, 17 aa, synthetic construct
KSSQSLLFSSNQKNYLA

SEQ ID NO: 14 - protein, 7 aa, synthetic construct
FASTRES

SEQ ID NO: 15 - protein, 9 aa, synthetic construct
QQHYRTPPT

SEQ ID NO: 16 - protein, 120 aa, synthetic construct
EITLKESGPTLVKPTQTLTLTCTFSGFSLSTYGIGVSWIRQPPGKALEWLAHIWWNDNKYYNTALKSRLTITKDTSKNQVVLTMTNMDPVDTATYYCARKEGSSAPFAYWGQGTLVTVSS

SEQ ID NO: 17 - protein, 113 aa, synthetic construct
DIVMTQSPDSLAVSLGERATINCKSSQSLLNSSNQKNYLAWYQQKPGQPPKLLIYFASTRESGVPDRFSGSGSGTDFTLTISLMQAEDVAVYYCQQHYRTPPTFGQGTKVEIK

SEQ ID NO: 18 - protein, 113 aa, synthetic construct
DIVMTQSPDSLAVSLGERATINCKSSQSLLFSSNQKNYLAWYQQKPGQPPKLLIYFASTRESGVPDRFSGSGSGTDFTLTISLMQAEDVAVYYCQQHYRTPPTFGQGTKVEIK

SEQ ID NO: 19 - DNA, 699 bp, synthetic construct
  source 1..699: mol_type = other DNA
gagatcaccctgaaggagagcggccccaccctggtgaagcccacccagaccctgaccctgacctgcaccttcagcggcttcagcctgagcacttatggtataggagtaagctggatcaggcagccccccggcaaggccctggagtggctggcccacatttggtggaatgataataagtactataacacagccctgaagagcaggctgaccatcaccaaggacaccagcaagaaccaggtggtgctgaccatgaccaacatggaccccgtggacaccgccacctactactgcgccaggaaggagggcagctcggccccctttgcttactggggccagggcaccctggtgaccgtgagcagcgacatcgtgatgacccagagccccgacagcctggccgtgagcctgggcgagagggccaccatcaactgcaagtccagtcagagccttttaaatagtagcaatcaaaagaactatttggcctggtaccagcagaagcccggccagccccccaagctgctgatctactttgcatccactagggaatctggcgtgcccgacaggttcagcggcagcggcagcggcaccgacttcaccctgaccatcagcagcctgcaggccgaggacgtggccgtgtactactgccagcaacattatagaactcctccgacgttcggccagggcaccaaggtggagatcaag

SEQ ID NO: 20 - DNA, 699 bp, synthetic construct
  source 1..699: mol_type = other DNA
gagatcaccctgaaggagagcggccccaccctggtgaagcccacccagaccctgaccctgacctgcaccttcagcggcttcagcctgagcacttatggtataggagtaagctggatcaggcagccccccggcaaggccctggagtggctggcccacatttggtggaatgataataagtactataacacagccctgaagagcaggctgaccatcaccaaggacaccagcaagaaccaggtggtgctgaccatgaccaacatggaccccgtggacaccgccacctactactgcgccaggaaggagggcagctcggccccctttgcttactggggccagggcaccctggtgaccgtgagcagcgacatcgtgatgacccagagccccgacagcctggccgtgagcctgggcgagagggccaccatcaactgcaagtccagtcagagccttttattcagtagcaatcaaaagaactatttggcctggtaccagcagaagcccggccagccccccaagctgctgatctactttgcatccactagggaatctggcgtgcccgacaggttcagcggcagcggcagcggcaccgacttcaccctgaccatcagcagcctgcaggccgaggacgtggccgtgtactactgccagcaacattatagaactcctccgacgttcggccagggcaccaaggtggagatcaag